European Patent Specification EP 3 762 499 B1, published December 20, 2023. Title: Reduction in Acetate Production by Yeast Over-Expressing PAB1. Applicant: Danisco US Inc. The sequence listing filed with the application follows.

SEQUENCE LISTING (4 sequences)

SEQ ID NO: 1 - protein, 577 aa, Saccharomyces cerevisiae
MADITDKTAEQLENLNIQDDQKQAATGSESQSVENSSASLYVGDLEPSVSEAHLYDIFSPIGSVSSIRVCRDAITKTSLGYAYVNFNDHEAGRKAIEQLNYTPIKGRLCRIMWSQRDPSLRKKGSGNIFIKNLHPDIDNKALYDTFSVFGDILSSKIATDENGKSKGFGFVHFEEEGAAKEAIDALNGMLLNGQEIYVAPHLSRKERDSQLEETKAHYTNLYVKNINSETTDEQFQELFAKFGPIVSASLEKDADGKLKGFGFVNYEKHEDAVKAVEALNDSELNGEKLYVGRAQKKNERMHVLKKQYEAYRLEKMAKYQGVNLFVKNLDDSVDDEKLEEEFAPYGTITSAKVMRTENGKSKGFGFVCFSTPEEATKAITEKNQQIVAGKPLYVAIAQRKDVRRSQLAQQIQARNQMRYQQATAAAAAAAAGMPGQFMPPMFYGVMPPRGVPFNGPNPQQMNPMGGMPKNGMPPQFRNGPVYGVPPQGGFPRNANDNNQFYQQKQRQALGEQLYKKVSAKTSNEEAAGKITGMILDLPPQEVFPLLESDELFEQHYKEASAAYESFKKEQEQQTEQA

SEQ ID NO: 2 - DNA, 1734 bp, Artificial Sequence
  synthetic construct
atggctgacatcaccgacaagactgccgaacaattggaaaacttgaacattcaagacgatcagaagcaagctgccactggttccgaatctcaatccgtcgaaaactcttccgcttctttgtacgttggtgacttagaaccatctgtctccgaagctcacttgtacgacatcttctctccaatcggttccgtctcttccatcagagtttgtcgtgatgctatcaccaagaccagcttgggttacgcttacgtcaactttaacgaccatgaagctggcagaaaggctatcgaacaattgaactacactccaatcaagggtagactatgtagaatcatgtggtctcaacgtgatccatccttgagaaagaaaggttctggcaacatcttcatcaagaacttgcatccagacattgacaacaaggctttgtacgatactttcagtgtctttggtgacatcttatcttccaagattgctaccgacgaaaacggaaagtccaagggttttggctttgttcacttcgaagaggaaggtgctgccaaggaagctatcgatgctttgaatggtatgctattgaacggtcaagaaatctacgttgctcctcacttgtccagaaaggaacgtgactctcaattggaagagaccaaggctcactacaccaacttgtacgtcaagaatatcaactccgaaactaccgacgaacaatttcaagaattgtttgccaagtttggtccaattgtttctgcttccttggaaaaggatgccgacggcaagttgaagggtttcggtttcgtcaactacgaaaagcacgaagacgctgtcaaggctgtcgaagccttgaacgattccgaactaaatggcgaaaagttgtacgttggtagagcacagaaaaagaacgaacgtatgcacgtcttgaagaaacaatacgaagcttacagattggaaaagatggccaagtaccaaggtgttaatttgttcgtcaagaacttggacgattctgtcgatgacgaaaagttggaagaggaatttgctccatacggtactatcacctctgccaaggtcatgagaaccgaaaacggtaagtccaagggttttggcttcgtctgtttctctactccagaggaagctaccaaggctatcaccgaaaagaatcaacagattgttgctggcaagccattgtacgttgccattgctcaaagaaaggacgtcagacgttctcaactagctcaacagatccaagccagaaaccaaatgagataccaacaggctactgctgccgctgcagctgccgctgcaggtatgccaggtcaattcatgcctccaatgttttacggtgtcatgcctccaagaggtgttccattcaacggtccaaaccctcaacagatgaatccaatgggtggaatgccaaagaacggtatgcctccacaattcagaaacggtccagtctacggtgtccctccacaaggtggctttccaagaaacgctaacgacaacaatcaattctaccaacagaagcaaagacaagctttgggtgaacaattgtacaagaaagtttctgccaagacttccaacgaagaagctgcaggcaagatcactggtatgatcttggatttaccacctcaagaagtcttcccactattggaatccgacgaattgttcgaacaacactacaaggaggcttctgctgcctacgaatctttcaaaaaggaacaagagcaacagactgaacaagcctaa

SEQ ID NO: 3 - DNA, 780 bp, Artificial Sequence
  synthetic construct
tatgttgtacctaaatcaataccgacagcttttgacatattatctgttatttacttgaatttttgtttcttgtaatacttgattacttttcttttgatgtgcttatcttacaaatagagaaaataaaacaacttaagtaagaattgggaaacgaaactacaactcaatcccttctcgaagatacatcaatccaccccttatataaccttgaagtcctcgaaacgatcagctaatctaaatggccccccttctttttgggttctttctctccctcttgccgccgatggaacgttctggaaaaagaagaataatttaattactttctcaactaaaatctggagaaaaaacgcaaatgacagcttctaaacgttccgtgtgctttctttctagaatgttctggaaagtttacaacaatccacaagaacgaaaatgccgttgacaatgatgaaaccatcatccacacaccgcgcacacgtgctttatttctttttctgaattttttttttccgccattttcaaccaaggaaattttttttcttagggctcagaacctgcaggtgaagaagcgctttagaaatcaaagcacaacgcaacaatttgtcgacaaccgagcctttgaagaaaaaatttttcacattgtcgcctctaaataaatagtttaaggttatctacccactatatttagttggttcttttttttttccttctactctttatctttttacctcatgctttctacctttcagcactgaagagtccaaccgaatatatacacacata

SEQ ID NO: 4 - DNA, 389 bp, Artificial Sequence
  synthetic construct
attaatataattatataaaaatattatcttcttttctttatatctagtgttatgtaaaataaattgatgactacggaaagcttttttatattgtttctttttcattctgagccacttaaatttcgtgaatgttcttgtaagggacggtagatttacaagtgatacaacaaaaagcaaggcgctttttctaataaaaagaagaaaagcatttaacaattgaacacctctatatcaacgaagaatattactttgtctctaaatccttgtaaaatgtgtacgatctctatatgggttactcataagtgtaccgaagactgcattgaaagtttatgttttttcactggaggcgtcattttcgcgttgagaagatgttcttatccaaatttcaa